European Patent Application EP 4 567 044 A1, published June 11, 2025. Title: High-stability recombinant collagen, and construction method thereof and use thereof. Applicant: Jiangsu Trautec Medical Technology Co, LTD. Application CN PCT/CN2023/111028, filed August 3, 2023. The sequence listing filed with the application follows.

SEQUENCE LISTING (10 sequences)

SEQ ID NO: 1 - protein, 474 aa, synthetic construct
  source 1..474: note = Amino acid sequence of original collagen
AGNTGAPGSPGVSGPKGDAGQPGEKGSPGAQGPPGAPGPLGIAGITGARGLAGPPGMPGPRGSPGPQGVKGESGKPGANGLSGERGPPGPQGLPGLAGTAGEPGRDGNPGSDGLPGRDGSPGGKGDRGENGSPGAPGAPGHPGPPGPVGPAGKSGDRGESGPAGPAGAPGPAGSRGAPGPQGPRGDKGETGERGAAGIKGHRGFPGNPGAPGSPGPAGQQGAIGSPGPAEFTAGNTGAPGSPGVSGPKGDAGQPGEKGSPGAQGPPGAPGPLGIAGITGARGLAGPPGMPGPRGSPGPQGVKGESGKPGANGLSGERGPPGPQGLPGLAGTAGEPGRDGNPGSDGLPGRDGSPGGKGDRGENGSPGAPGAPGHPGPPGPVGPAGKSGDRGESGPAGPAGAPGPAGSRGAPGPQGPRGDKGETGERGAAGIKGHRGFPGNPGAPGSPGPAGQQGAIGSPGPADHHHHHHTGLARF

SEQ ID NO: 2 - protein, 463 aa, synthetic construct
  source 1..463: note = Amino acid sequence of recombinant collagen variant M2
AGNTGAPGSPGVSGPKGDAGQPGEKGSPGAQGPPGAPGPSGPAGITGARGPAGPPGMPGPRGSPGPQGVKGESGKPGAQGLSGERGPPGPQGLPGPAGTAGEPGRDGNPGSDGLPGRDGSPGGKGERGEQGSPGAPGAPGHPGPPGPVGPAGKSGERGESGPAGPAGAPGPAGSRGAPGPQGPRGDKGETGERGPAGEKGHRGPPGNPGAPGSPGPAGQQGAIGSPGPAGNTGAPGSPGVSGPKGDAGQPGEKGSPGAQGPPGAPGPSGPAGITGARGPAGPPGMPGPRGSPGPQGVKGESGKPGAQGLSGERGPPGPQGLPGPAGTAGEPGRDGNPGSDGLPGRDGSPGGKGERGEQGSPGAPGAPGHPGPPGPVGPAGKSGERGESGPAGPAGAPGPAGSRGAPGPQGPRGDKGETGERGPAGEKGHRGPPGNPGAPGSPGPAGQQGAIGSPGPAHHHHHH

SEQ ID NO: 3 - protein, 457 aa, synthetic construct
  source 1..457: note = Amino acid sequence of recombinant collagen variant M4
AGNTGAPGSPGVSGPKGDAGQPGEKGSPGAQGPPGAPGPSGPAGITGAKGPAGPPGMPGPKGSPGPQGVKGESGKPGAQGLSGEKGPPGPQGLPGPAGTAGEPGKDGNPGSDGLPGKDGSPGGKGEKGENGSPGAPGAPGHPGPPGPVGPAGKSGEKGESGPAGPAGAPGPAGSKGAPGPQGPRGDKGETGEKGPAGEKGHRGPPGNPGAPGSPGPAGQQGAIGSPGPAGNTGAPGSPGVSGPKGDAGQPGEKGSPGAQGPPGAPGPSGPAGITGAKGPAGPPGMPGPKGSPGPQGVKGESGKPGAQGLSGEKGPPGPQGLPGPAGTAGEPGKDGNPGSDGLPGKDGSPGGKGEKGENGSPGAPGAPGHPGPPGPVGPAGKSGEKGESGPAGPAGAPGPAGSKGAPGPQGPRGDKGETGEKGPAGEKGHRGPPGNPGAPGSPGPAGQQGAIGSPGPA

SEQ ID NO: 4 - protein, 463 aa, synthetic construct
  source 1..463: note = Amino acid sequence of recombinant collagen variant M5
AGNTGAPGSPGVSGPKGEAGQPGEKGSPGAQGPPGAPGPSGPAGITGARGDAGPPGPPGPRGSPGPQGVKGESGKPGAQGLSGERGDPGPQGLPGPAGTAGEPGREGNPGSEGLPGREGSPGGKGERGDQGSPGAPGAPGHPGPPGPVGPAGKSGERGESGPAGPAGAPGPAGSRGAPGPQGPRGDKGETGERGPAGEKGHRGPPGNPGAPGSPGPAGQQGAIGSPGPAGNTGAPGSPGVSGPKGEAGQPGEKGSPGAQGPPGAPGPSGPAGITGARGDAGPPGPPGPRGSPGPQGVKGESGKPGAQGLSGERGDPGPQGLPGPAGTAGEPGREGNPGSEGLPGREGSPGGKGERGDQGSPGAPGAPGHPGPPGPVGPAGKSGERGESGPAGPAGAPGPAGSRGAPGPQGPRGDKGETGERGPAGEKGHRGPPGNPGAPGSPGPAGQQGAIGSPGPAHHHHHH

SEQ ID NO: 5 - protein, 99 aa, synthetic construct
  source 1..99: note = Amino acid sequence of a monomer formed by selecting and splicing sequences without MMP cleavage site and unstable triplet in the original sequence
GNTGAPGSPGVSGPKGDAGQPGEKGSPGAQGPPGAPGSPGPQGVKGESGKPGANGLSGENGSPGAPGAPGHPGPPGPVGPAGKSGAPGPQGPRGDKGET

SEQ ID NO: 6 - protein, 500 aa, synthetic construct
  source 1..500: note = Amino acid sequence of recombinant collagen variant M6
GPPGNTGAPGSPGVSGPKGDAGQPGEKGSPGAQGPPGAPGSPGPQGVKGESGKPGANGLSGENGSPGAPGAPGHPGPPGPVGPAGKSGAPGPQGPRGDKGETGNTGAPGSPGVSGPKGDAGQPGEKGSPGAQGPPGAPGSPGPQGVKGESGKPGANGLSGENGSPGAPGAPGHPGPPGPVGPAGKSGAPGPQGPRGDKGETGNTGAPGSPGVSGPKGDAGQPGEKGSPGAQGPPGAPGSPGPQGVKGESGKPGANGLSGENGSPGAPGAPGHPGPPGPVGPAGKSGAPGPQGPRGDKGETGNTGAPGSPGVSGPKGDAGQPGEKGSPGAQGPPGAPGSPGPQGVKGESGKPGANGLSGENGSPGAPGAPGHPGPPGPVGPAGKSGAPGPQGPRGDKGETGNTGAPGSPGVSGPKGDAGQPGEKGSPGAQGPPGAPGSPGPQGVKGESGKPGANGLSGENGSPGAPGAPGHPGPPGPVGPAGKSGAPGPQGPRGDKGETGG

SEQ ID NO: 7 - DNA, 1392 bp, synthetic construct
  source 1..1392: mol_type = other DNA; note = Polynucleotide sequence encoding the recombinant collagen variant M2
gctggtaacactggtgctccaggttctcctggtgtttctggtccaaagggagatgctggtcaaccaggtgaaaaaggttctcctggtgctcaaggtccacctggtgctccaggtccttctggtccagctggtattactggtgctagaggtcctgccggtccacctggtatgccaggtcctagaggttctccaggtcctcaaggtgttaagggtgaatctggtaaaccaggtgctcaaggtttgtccggagagagaggtccacctggtccacaaggtttgccaggtcctgctggtactgctggagagccaggtagagatggtaatcctggttctgatggtttgccaggtagagatggttctccaggtggtaaaggtgaaagaggtgagcaaggttctccaggtgctcctggtgctccaggtcatccaggtccacctggaccagttggtcctgctggtaaatctggtgaaagaggtgagtctggtccagctggtcctgctggtgctccaggtcctgctggttctagaggtgctccaggtcctcaaggtccaagaggagataagggtgaaactggagagagaggtcctgctggtgaaaaaggtcacagaggtccacctggtaacccaggtgctcctggttctccaggtcctgctggtcaacaaggtgctatcggttctcctggtcctgctggtaataccggtgctccaggttctccaggtgtttctggacctaaaggagatgccggtcaaccaggagagaagggttctccaggtgctcaaggtccacctggtgctccagggccatccggacctgccggaatcaccggtgctagaggaccagccggtccacctggaatgcctggaccaagaggttctcctggaccacagggagtcaaaggagagtccggtaaacctggtgctcaaggactttccggagaaagaggtccacctggacctcagggacttcctggaccagctggtactgctggtgaaccaggtagagatggtaacccaggttctgacggacttcctggaagagacggttctccaggtggtaaaggggagagaggtgagcagggttctcctggtgctcctggtgctccagggcacccaggtccacctggacctgtcggaccagccggtaaatccggagagagaggtgagtccggacctgccggaccagccggtgctccaggaccagccggttctagaggtgctccagggccacagggacctagaggagataaaggagagaccggagagagaggtccagccggagagaagggacatagaggtccacctggtaatcctggtgctcctggttctcctggaccagccggacaacaaggtgctattggttctcctggacctgctcatcaccatcaccatcactaa

SEQ ID NO: 8 - DNA, 1371 bp, synthetic construct
  source 1..1371: mol_type = other DNA; note = Polynucleotide sequence encoding the recombinant collagen variant M4
gcaggtaacactggtgcgcccggctcgcctggcgtaagtggtccaaaaggggatgctggtcagcccggggaaaagggatctcccggagcacaaggacctcccggggcgcccggtcctagcggccctgcaggaattactggtgctaaggggccagctggcccgccgggtatgcctggacccaaagggtcaccaggcccacagggagtcaaaggagaatccggcaagccgggagcgcaagggctgtccggtgagaaaggaccacctggaccccagggactaccagggccagccggtaccgctggcgagccggggaaagatgggaaccctgggagtgacggattaccggggaaagacgggagccccggtggcaagggcgagaagggtgagaacggctcaccgggggctcccggagctccgggtcacccggggccgccagggccagtagggccagccgggaagtcgggggagaaaggagaatcaggacccgccggcccggctggagcacccggaccagctggaagcaaaggagcgccagggccacaggggcctagaggggacaagggtgaaacaggtgaaaaggggccggcgggagaaaaaggtcatcgaggtcccccgggaaatccaggtgctcctggatcgcctggtccggcgggtcaacagggtgcaatcggaagtccgggccctgcaggcaatacgggagctcccggctcccccggagtgtctggtcccaagggtgatgccgggcaaccgggcgagaaggggtcacctggtgcgcagggaccccctggtgccccaggccccagtggtcccgccggcatcacaggggcaaaaggccctgctggacccccaggaatgccggggccgaagggatcacctggaccacagggggttaagggcgaatccggcaaacccggagcacaaggtctctcgggcgaaaaaggaccgcctgggcctcaaggtcttccgggacccgcaggcacggccggggaaccgggaaaagacggaaatccagggtcggatggtttgccaggcaaagacggttctcccggcggcaagggcgagaagggggagaatggcagcccaggcgcgcccggagccccaggtcatccaggcccgcctgggccagtcggtcctgcaggcaaaagtggcgagaagggtgagtctgggcctgccgggcctgccggcgccccaggtcccgccggttctaagggcgcgcccggaccgcaaggcccgcgtggtgataagggggagaccggcgaaaaaggccctgcgggcgaaaaaggacaccgcgggccacctgggaacccgggtgcgccgggtagccctggtcctgcaggccagcaaggcgctatagggtccccgggtcctgca

SEQ ID NO: 9 - DNA, 1389 bp, synthetic construct
  source 1..1389: mol_type = other DNA; note = Polynucleotide sequence encoding the recombinant collagen variant M5
gctgggaacactggggcgcctggcagtcctggagtatccggcccgaaaggagaggccggccagcctggggagaagggaagcccaggggctcaaggaccaccgggggcccccggaccgagtggtccagcggggattactggagctaggggagatgccgggcctccgggtccgcccggtccccggggttcgccaggcccgcaaggagtgaagggagagagtggtaaaccgggggcacaaggtttatctggtgaaaggggagaccctgggccgcagggtctccctggtccagccgggacggcaggagagcctgggagagagggaaaccccgggagcgaaggattgcctggtcgtgaaggctcacccggcggcaagggtgagcgcggtgaccaaggctcgccgggagcaccgggtgctcctggccaccccgggcctccagggccagtcgggccagccggtaagtcaggggagagaggagagtctgggccagcgggcccggcaggtgcgcccggtccagccggaagtcgcggtgcaccgggccctcaaggtccgagaggggataagggcgagacaggagagcggggtccggcgggggaaaagggacatcgcggccctccgggaaatccaggtgctccagggtctcccggtcctgctgggcagcagggtgcaataggttctccaggccctgccgggaataccggcgcgccaggatcgccaggagtctcgggtcccaaaggggaggccggccaacccggggaaaaaggctcacccggcgcgcaaggcccgcccggcgctcctggacccagtggacccgccggtatcacgggtgcaaggggggacgccggtccaccaggaccccctggtcctcgaggcagcccaggaccccagggagttaagggagaatcaggcaaacctggcgctcaaggtctgtctggcgagaggggcgatccaggtccgcaggggcttccgggtcccgcaggtacagctggagaacccgggcgagaaggaaatccaggaagcgaaggactacctggacgggaagggagcccggggggaaagggcgaacgtggcgatcagggctccccaggcgcaccgggggcgccaggtcatcctggacctcccggccctgtaggacccgcgggtaaatccggagaacgtggcgaatccggcccggcggggcccgctggtgccccaggacccgccgggtcgcgcggggctcctgggccccaaggtcctcgaggcgacaagggggagaccggcgaacgtggtcctgctggtgagaaaggtcaccgaggcccgccgggcaaccctggggcaccggggtcccccgggccagcgggccagcagggcgcgatcgggtcaccaggaccggcacatcaccaccatcatcac

SEQ ID NO: 10 - DNA, 1500 bp, synthetic construct
  source 1..1500: mol_type = other DNA; note = Polynucleotide sequence encoding the recombinant collagen variant M6
gggccgccaggtaataccggtgcgcctgggtccccgggagtttcaggtcctaaaggcgaggcggggcaaccgggagagaaaggaagtcccggggctcagggcccgccgggtgccccgggtagccccggtcctcagggtgtaaagggtgagagcgggaagcctggcgcacaaggtttgagcggcgagcaaggctcacctggagcccccggtgcacccgggcacccgggtcctcctgggccggtaggaccagcaggaaaatcaggtgcgccagggcctcaaggtccccgaggtgacaaaggggaaaccgggaatactggcgctccgggctcgccaggggtttcaggtcctaagggggaagctgggcagccgggcgaaaagggctcgcccggtgcacagggcccgccaggagcgcccgggtcgcccggtccccagggcgtcaaaggagagagcggcaagcctggggcccagggactttctggcgaacaaggaagtcctggggctcctggagcccctggtcaccccggtccccccggaccagtcggccctgcaggtaaatctggagcgccaggaccgcagggaccacggggggataagggcgaaacaggaaataccggtgctccaggttctccaggggttagcggcccgaagggtgaagcgggccaacccggtgagaaaggatcgccgggcgcccagggcccgccgggtgcccccggctcacccggaccgcaaggcgtcaaaggagagtcggggaaaccaggtgcccaaggtctgtccggggaacaaggaagtccaggcgcaccgggtgctcctggacatccaggcccccctggccccgttggtcctgcgggtaaatccggcgctcccgggcctcaaggacctaggggggacaagggagagacgggcaacacgggcgccccagggtctcctggagtgtctgggcccaagggggaggcgggtcaacccggggaaaaaggttctcctggtgctcaaggccccccgggcgctccaggctcgccggggccgcagggagtaaagggcgagagtggaaagcctggagcccagggattatcgggtgagcaaggatcacccggcgcgccaggggcgccgggccaccctggacctccaggtccagtggggccagcgggtaaaagcggcgcaccagggccgcaggggccccgtggggataaaggagaaacagggaacactggtgcgccgggttccccgggcgtcagtgggcccaagggggaagctggacagccaggagaaaaaggttctccaggagcacagggtcccccaggggcaccaggttctcctggcccacagggagtgaagggagaatcagggaaacctggcgcacaggggctcagtggtgaacaaggaagccccggggcccctggggccccggggcatccaggccctcccggcccggtaggcccggcaggtaaatccggggctcctggtccccaaggccctagaggggataagggcgagactggagga